European Patent Specification EP 3 965 738 B1, published August 6, 2025. Title: METHOD FOR PRODUCTION OF LIPOSOMES. Applicant: UNIVERSIDADE DO MINHO. The sequence listing filed with the application follows.

SEQUENCE LISTING (3 sequences)

SEQ ID NO: 1 - protein, 12 aa, Artificial Sequence
  Folic Acid with SEQ ID 1
DRDDQAAWFSQY

SEQ ID NO: 2 - protein, 43 aa, Artificial Sequence
  Sequence 2
KDEPQRRSARLSAKPAPPKPEPKPKKAPAKKDRDDQAAWFSQY

SEQ ID NO: 3 - protein, 43 aa, Artificial Sequence
  Sequence 3
YQSFWAAQDDRDKDEPQRRSARLSAKPAPPKPEPKPKKAPAKK